European Patent Application EP 4 356 924 A2, published April 24, 2024. Title: Human Monoclonal Antibodies to Severe Acute Respiratory Syndrome Coronavirus 2 (SARS-CoV-2). Applicant: Vanderbilt University. The sequence listing filed with the application follows.

SEQUENCE LISTING (187 sequences)

SEQ ID NO: 1 - DNA, 351 bp, synthetic construct
  misc_feature 1..351: note = COV2-2165 Heavy
  source 1..351: mol_type = other DNA
gaggtgcagctggtggagtctgggggaggcttggtccagcctggggggtctctgagactctcctgtgcagcctctggactcaccgtccgtagcaactacatgacctgggtccgccagactccagggaaggggctggaatgggtgtcagttatttatagcggtggtagcacattctacgcagactccgtgaagggcagattcaccatctccagagacaattccaagaacacggtgtatcttcaaatgaacagcctgagagccgaggacacggctgtgtattactgtgcgagagatctcgtgacttacggtttggacgtctggggccaagggaccacggtcaccgtctcctca

SEQ ID NO: 2 - DNA, 321 bp, synthetic construct
  misc_feature 1..321: note = COV2-2165 Light
  source 1..321: mol_type = other DNA
gacatccagttgacccagtctccatccttcctgtctgcatctgtaggagacagagtcaccatcacttgccgggccagtcagggcattagcaattatttagcctggtatcagcaaaaaccagggacagcccctaacctcctgatctatgctgcatccactttgcaaagtggggtcccatcaaggttcagcggcagtggatctgggacagaattcactctcacaatcagcagcctgcagcctgaagattttgcaacttattactgtcaactacttaatagtcaccccctcaccttcggccaagggacacgactggagattaaa

SEQ ID NO: 3 - DNA, 370 bp, synthetic construct
  misc_feature 1..370: note = COV2-2838 Heavy
  source 1..370: mol_type = other DNA
caaatgcagctggtgcagtctgggcctgaggtgaagaagcctgggacctcagtgaaggtctcctgcaaggcttctggattcacctttatgagctctgctgtgcagtgggtgcgacaggctcgtggacaacgccttgagtggataggatggatcgtcattggcagtggtaacacaaactacgcacagaagttccaggaaagagtcaccattaccagggacatgtccacaagcacagcctacatggagctgagcagcctgagatccgaggacacggccgtgtattactgtgcggccccatattgtagtagtatcagctgcaatgatggttttgatatctggggccaagggacaatggtcaccgtctcttcag

SEQ ID NO: 4 - DNA, 328 bp, synthetic construct
  misc_feature 1..328: note = COV2-2838 Light
  source 1..328: mol_type = other DNA
gaaattgtgttgacgcagtctccaggcaccctgtctttgtctccaggggagagagccaccctctcctgcagggccagtcagagtgttagcagcagctacttagcctggtaccagcagaaacctggccaggctcccaggctcctcatctatggtgcatccagcagggccactggcatcccagacaggttcagtggcagtgggtctgggacagacttcactctcaccatcagcagactggagcctgaagattttgcagtgtattactgtcagcactatggtagctcacggggttggacgttcggccaagggaccaaggtggaaatcaaac

SEQ ID NO: 5 - DNA, 351 bp, synthetic construct; identical to SEQ ID NO: 1
  misc_feature 1..351: note = COV2-2952 heavy
  source 1..351: mol_type = other DNA

SEQ ID NO: 6 - DNA, 322 bp, synthetic construct
  misc_feature 1..322: note = COV2-2952 light
  source 1..322: mol_type = other DNA
gacatccagttgacccagtctccatccttcctgtctgcatctgtaggagacagagtcaccatcacttgccgggccagtcagggcattagcaattatttagcctggtatcagcaaaaaccagggacagcccctaacctcctgatctatgctgcatccactttgcaaagtggggtcccatcaaggttcagcggcagtggatctgggacagaattcactctcacaatcagcagcctgcagcctgaagattttgcaacttattactgtcaactacttaatagtcaccccctcaccttcggccaagggacacgactggagattaaac

SEQ ID NO: 7 - DNA, 388 bp, synthetic construct
  misc_feature 1..388: note = COV2-2514 heavy
  source 1..388: mol_type = other DNA
gaggtgcagctggtggagtctgggggaggtgtggtacggcctggggggtccctgagactctcctgtgcagcctctggattcatctttgatgattatgacatgacctgggtccgccaagctccagggaaggggctggagtgggtctctggtattaattggaatggtggtagcacaggttatgcagactctgtgaagggccgattcaccatctccagagacaacgccaagaactccctgtatctgcaaatgaacagtctgagagccgaggacacggccttgtatcactgtgcagtgattatgtctccaatcccccgttatagtggctacgattgggcgggtgatgcttttgatatctggggccaagggacaatggtcaccgtctcttcag

SEQ ID NO: 8 - DNA, 325 bp, synthetic construct
  misc_feature 1..325: note = COV2-2514 light
  source 1..325: mol_type = other DNA
tcttctgagctgactcaggaccctgctgtgtctgtggccttgggacagacagtcaggatcacatgccaaggagacagcctcagaagctattatgcaagttggtaccagcagaagccaggacaggtccctatacttgtcatctatgataaaaacaaccggccctcagggatcccagaccgattctctggctccagctcaggaaacacagcttccttgaccatcactggggctcaggcggaagatgaggctgactattactgtaactcccgggacagcagtggtaacgccgtggtattcggcggagggaccaagctgaccgtcctag

SEQ ID NO: 9 - DNA, 370 bp, synthetic construct
  misc_feature 1..370: note = COV2-2391 heavy
  source 1..370: mol_type = other DNA
caggtgcagctggtgcagtctggggctgaggtgaagaagcctggggcctcagtgaaggtctcctgcaaggcttctggatacaccttcggcagctttgatatcaactgggtgcgacaggccactggacaagggcttgagtggatgggacggatgaactctaacagtgggaacacagcctatgcacagaagttccagggcagagtcactatgaccagggacacctccacaaatacagcctacatggagttgagcagcctgagatctgaggacacggccatgtattactgtgcgagaatgcgcagtggctggcccacacatggccgcccggatgacttctggggccggggaaccctggtcaccgtctcctcag

SEQ ID NO: 10 - DNA, 331 bp, synthetic construct
  misc_feature 1..331: note = COV2-2391 light
  source 1..331: mol_type = other DNA
cagtctgtgctgactcaggcaccctcagcgtctgggacccccgggcagagggtcaccatctcttgttctggaagcaactccaatatcggaagttatactataaactggtaccagcagctcccaggaacggcccccaaactcctcatttatggtaatgatcagcggacctcaggggtccctgaccgattctctggctccaagtttggcacctcggcctccctggccatcagtgggctccagtctgaggatgaaaataattattactgtgcagtatgggatgacagcctgaatggcctggtattcggcggagggaccaaactgaccgtcctag

SEQ ID NO: 11 - DNA, 369 bp, synthetic construct
  misc_feature 1..369: note = COV2-3025 heavy
  source 1..369: mol_type = other DNA
gaggtgcagctggtgcagtctgggcctgaggtgaagaagcctgggacctcagtgaaggtctcctgcaaggcttctggattcacctttatgagctctgctgtgcagtgggtgcgacaggctcgtggacaacgccttgagtggataggatggatcgtcattggcagtggtaacacaaactacgcacagaagttccaggaaagagtcaccattaccagggacatgtccacaagcacagcctacatggagctgagcagcctgagatccgaggacacggccgtgtattactgtgcggccccatattgtagtagtatcagctgcaatgatggttttgatatctggggccaagggacaatggtcaccgtctcttca

SEQ ID NO: 12 - DNA, 327 bp, synthetic construct
  misc_feature 1..327: note = COV2-3025 light
  source 1..327: mol_type = other DNA
gaaattgtgttgacgcagtctccaggcaccctgtctttgtctccaggggagagagtcaccctctcctgcagggccagtcagagtgttagcagcagctacttagcctggtaccagcagaaacctggccaggctcccaggctcctcatctatggtgcatccagcagggccactggcatcccagacaggttcagtggcagtgggtctgggacagacttcactctcaccatcagcagactggagcctgaagattttgcagtgtattactgtcagcactatggtagctcacggggttggacgttcggccaagggaccaaggtggaaatcaaa

SEQ ID NO: 13 - DNA, 369 bp, synthetic construct
  misc_feature 1..369: note = COV2-2196 heavy
  source 1..369: mol_type = other DNA
caaatgcagctggtgcagtctgggcctgaggtgaagaagcctgggacctcagtgaaggtctcctgcaaggcttctggattcacctttatgagctctgctgtgcagtgggtgcgacaggctcgtggacaacgccttgagtggataggatggatcgtcattggcagtggtaacacaaactacgcacagaagttccaggaaagagtcaccattaccagggacatgtccacaagcacagcctacatggagctgagcagcctgagatccgaggacacggccgtgtattactgtgcggccccatattgtagtagtatcagctgcaatgatggttttgatatctggggccaagggacaatggtcaccgtctcttca

SEQ ID NO: 14 - DNA, 327 bp, synthetic construct
  misc_feature 1..327: note = COV2-2196 light
  source 1..327: mol_type = other DNA
gaaattgtgttgacgcagtctccaggcaccctgtctttgtctccaggggagagagccaccctctcctgcagggccagtcagagtgttagcagcagctacttagcctggtaccagcagaaacctggccaggctcccaggctcctcatctatggtgcatccagcagggccactggcatcccagacaggttcagtggcagtgggtctgggacagacttcactctcaccatcagcagactggagcctgaagattttgcagtgtattactgtcagcactatggtagctcacggggttggacgttcggccaagggaccaaggtggaaatcaaa

SEQ ID NO: 15 - DNA, 387 bp, synthetic construct
  misc_feature 1..387: note = COV2-2094 heavy
  source 1..387: mol_type = other DNA
gaggtgcagctggtggagtctgggggaggtgtggtacggcctggggggtccctgagactctcctgtgcagcctctggattcatctttgatgattatgacatgacctgggtccgccaagctccagggaaggggctggagtgggtctctggtattaattggaatggtggtagcacaggttatgcagactctgtgaagggccgattcaccatctccagagacaacgccaagaactccctgtatctgcaaatgaacagtctgagagccgaggacacggccttgtatcactgtgcagtgattatgtctccaatcccccgttatagtggctacgattgggcgggtgatgcttttgatatctggggccaagggacaatggtcaccgtctcttca

SEQ ID NO: 16 - DNA, 324 bp, synthetic construct
  misc_feature 1..324: note = COV2-2094 light
  source 1..324: mol_type = other DNA
tcttctgagctgactcaggaccctgctgtgtctgtggccttgggacagacagtcaggatcacatgccaaggagacagcctcagaagctattatgcaagttggtaccagcagaagccaggacaggtccctatacttgtcatctatgataaaaacaaccggccctcagggatcccagaccgattctctggctccagctcaggaaacacagcttccttgaccatcactggggctcaggcggaagatgaggctgactattactgtaactcccgggacagcagtggtaacgccgtggtattcggcggagggaccaagctgaccgtccta

SEQ ID NO: 17 - DNA, 369 bp, synthetic construct
  misc_feature 1..369: note = COV2-2096 heavy
  source 1..369: mol_type = other DNA
caggtgcagctggtgcagtctggggctgaggtgaagaagcctggggcctcagtgaaggtctcctgcaaggcttctggatacaccttcggcagctttgatatcaactgggtgcgacaggccactggacaagggcttgagtggatgggacggatgaactctaacagtgggaacacagcctatgcacagaagttccagggcagagtcactatgaccagggacacctccacaaatacagcctacatggagttgagcagcctgagatctgaggacacggccatgtattactgtgcgagaatgcgcagtggctggcccacacatggccgcccggatgacttctggggccggggaaccctggtcaccgtctcctca

SEQ ID NO: 18 - DNA, 330 bp, synthetic construct
  misc_feature 1..330: note = COV2-2096 light
  source 1..330: mol_type = other DNA
cagtctgtgctgactcaggcaccctcagcgtctgggacccccgggcagagggtcaccatctcttgttctggaagcaactccaatatcggaagttatactataaactggtaccagcagctcccaggaacggcccccaaactcctcatttatggtaatgatcagcggacctcaggggtccctgaccgattctctggctccaagtttggcacctcggcctccctggccatcagtgggctccagtctgaggatgaaaataattattactgtgcagtatgggatgacagcctgaatggcctggtattcggcggagggaccaaactgaccgtccta

SEQ ID NO: 19 - DNA, 393 bp, synthetic construct
  misc_feature 1..393: note = COV2-2130 heavy
  source 1..393: mol_type = other DNA
gaggtgcagctggtggagtctgggggaggcttggtaaagcctggggggtcccttagactctcctgtgcagcctctggattcactttcagagacgtctggatgagctgggtccgccaggctccagggaaggggctggagtgggttggccgtattaaaagcaaaattgatggtgggacaacagactacgctgcacccgtgaaaggcagattcaccatctcaagagatgattcaaaaaacacgctgtatctgcaaatgaacagcctgaaaaccgaggacacagccgtgtattactgtaccacagcgggaagctattactatgatactgttggtccaggcctcccagagggaaaatttgactactggggccagggaaccctggtcaccgtctcctca

SEQ ID NO: 20 - DNA, 336 bp, synthetic construct
  misc_feature 1..336: note = COV2-2130 light
  source 1..336: mol_type = other DNA
gacatcgtgatgacccagtctccagactccctggctgtgtctctgggcgagagggccaccatcaactgcaagtccagccagagtgttttatacagctccaacaataagaactacttagcttggtaccagcagaaaccaggacagcctcctaagctgctcatgtactgggcatctacccgggaatccggggtccctgaccgattcagtggcagcgggtctggggcagagttcactctcaccatcagcagcctgcaggctgaagatgtggcaatttattactgtcagcaatattatagtaccctcactttcggcggagggaccaaggtggagatcaaa

SEQ ID NO: 21 - protein, 117 aa, synthetic construct
  REGION 1..117: note = COV2-2165 heavy
EVQLVESGGGLVQPGGSLRLSCAASGLTVRSNYMTWVRQTPGKGLEWVSVIYSGGSTFYADSVKGRFTISRDNSKNTVYLQMNSLRAEDTAVYYCARDLVTYGLDVWGQGTTVTVSS

SEQ ID NO: 22 - protein, 107 aa, synthetic construct
  REGION 1..107: note = COV2-2165 light
DIQLTQSPSFLSASVGDRVTITCRASQGISNYLAWYQQKPGTAPNLLIYAASTLQSGVPSRFSGSGSGTEFTLTISSLQPEDFATYYCQLLNSHPLTFGQGTRLEIK

SEQ ID NO: 23 - protein, 123 aa, synthetic construct
  REGION 1..123: note = COV2-2838 heavy
QMQLVQSGPEVKKPGTSVKVSCKASGFTFMSSAVQWVRQARGQRLEWIGWIVIGSGNTNYAQKFQERVTITRDMSTSTAYMELSSLRSEDTAVYYCAAPYCSSISCNDGFDIWGQGTMVTVSS

SEQ ID NO: 24 - protein, 109 aa, synthetic construct
  REGION 1..109: note = COV2-2838 light
EIVLTQSPGTLSLSPGERATLSCRASQSVSSSYLAWYQQKPGQAPRLLIYGASSRATGIPDRFSGSGSGTDFTLTISRLEPEDFAVYYCQHYGSSRGWTFGQGTKVEIK

SEQ ID NO: 25 - protein, 117 aa, synthetic construct; identical to SEQ ID NO: 21
  REGION 1..117: note = COV2-2952 heavy

SEQ ID NO: 26 - protein, 107 aa, synthetic construct; identical to SEQ ID NO: 22
  REGION 1..107: note = COV2-2952 light

SEQ ID NO: 27 - protein, 129 aa, synthetic construct
  REGION 1..129: note = COV2-2514 heavy
EVQLVESGGGVVRPGGSLRLSCAASGFIFDDYDMTWVRQAPGKGLEWVSGINWNGGSTGYADSVKGRFTISRDNAKNSLYLQMNSLRAEDTALYHCAVIMSPIPRYSGYDWAGDAFDIWGQGTMVTVSS

SEQ ID NO: 28 - protein, 108 aa, synthetic construct
  REGION 1..108: note = COV2-2514 light
SSELTQDPAVSVALGQTVRITCQGDSLRSYYASWYQQKPGQVPILVIYDKNNRPSGIPDRFSGSSSGNTASLTITGAQAEDEADYYCNSRDSSGNAVVFGGGTKLTVL

SEQ ID NO: 29 - protein, 123 aa, synthetic construct
  REGION 1..123: note = COV2-2391 heavy
QVQLVQSGAEVKKPGASVKVSCKASGYTFGSFDINWVRQATGQGLEWMGRMNSNSGNTAYAQKFQGRVTMTRDTSTNTAYMELSSLRSEDTAMYYCARMRSGWPTHGRPDDFWGRGTLVTVSS

SEQ ID NO: 30 - protein, 110 aa, synthetic construct
  REGION 1..110: note = COV2-2391 light
QSVLTQAPSASGTPGQRVTISCSGSNSNIGSYTINWYQQLPGTAPKLLIYGNDQRTSGVPDRFSGSKFGTSASLAISGLQSEDENNYYCAVWDDSLNGLVFGGGTKLTVL

SEQ ID NO: 31 - protein, 123 aa, synthetic construct
  REGION 1..123: note = COV2-3025 heavy
EVQLVQSGPEVKKPGTSVKVSCKASGFTFMSSAVQWVRQARGQRLEWIGWIVIGSGNTNYAQKFQERVTITRDMSTSTAYMELSSLRSEDTAVYYCAAPYCSSISCNDGFDIWGQGTMVTVSS

SEQ ID NO: 32 - protein, 109 aa, synthetic construct
  REGION 1..109: note = COV2-3025 light
EIVLTQSPGTLSLSPGERVTLSCRASQSVSSSYLAWYQQKPGQAPRLLIYGASSRATGIPDRFSGSGSGTDFTLTISRLEPEDFAVYYCQHYGSSRGWTFGQGTKVEIK

SEQ ID NO: 33 - protein, 123 aa, synthetic construct; identical to SEQ ID NO: 23
  REGION 1..123: note = COV2-2196 heavy

SEQ ID NO: 34 - protein, 109 aa, synthetic construct; identical to SEQ ID NO: 24
  REGION 1..109: note = COV2-2196 light

SEQ ID NO: 35 - protein, 129 aa, synthetic construct; identical to SEQ ID NO: 27
  REGION 1..129: note = COV2-2094 heavy

SEQ ID NO: 36 - protein, 108 aa, synthetic construct; identical to SEQ ID NO: 28
  REGION 1..108: note = COV2-2094 light

SEQ ID NO: 37 - protein, 123 aa, synthetic construct; identical to SEQ ID NO: 29
  REGION 1..123: note = COV2-2096 heavy

SEQ ID NO: 38 - protein, 110 aa, synthetic construct; identical to SEQ ID NO: 30
  REGION 1..110: note = COV2-2096 light

SEQ ID NO: 39 - protein, 131 aa, synthetic construct
  REGION 1..131: note = COV2-2130 heavy
EVQLVESGGGLVKPGGSLRLSCAASGFTFRDVWMSWVRQAPGKGLEWVGRIKSKIDGGTTDYAAPVKGRFTISRDDSKNTLYLQMNSLKTEDTAVYYCTTAGSYYYDTVGPGLPEGKFDYWGQGTLVTVSS

SEQ ID NO: 40 - protein, 112 aa, synthetic construct
  REGION 1..112: note = COV2-2130 light
DIVMTQSPDSLAVSLGERATINCKSSQSVLYSSNNKNYLAWYQQKPGQPPKLLMYWASTRESGVPDRFSGSGSGAEFTLTISSLQAEDVAIYYCQQYYSTLTFGGGTKVEIK

SEQ ID NO: 41 - protein, 8 aa, synthetic construct
  REGION 1..8: note = COV2-2165 CDRH1
GLTVRSNY

SEQ ID NO: 42 - protein, 7 aa, synthetic construct
  REGION 1..7: note = COV2-2165 CDRH2
IYSGGST

SEQ ID NO: 43 - protein, 11 aa, synthetic construct
  REGION 1..11: note = COV2-2165 CDRH3
ARDLVTYGLDV

SEQ ID NO: 44 - protein, 8 aa, synthetic construct
  REGION 1..8: note = COV2-2838 CDRH1
GFTFMSSA

SEQ ID NO: 45 - protein, 8 aa, synthetic construct
  REGION 1..8: note = COV2-2838 CDRH2
IVIGSGNT

SEQ ID NO: 46 - protein, 16 aa, synthetic construct
  REGION 1..16: note = COV2-2838 CDRH3
AAPYCSSISCNDGFDI

SEQ ID NO: 47 - protein, 8 aa, synthetic construct
  REGION 1..8: note = COV2-2952 CDRH1
GLTVRSNY

SEQ ID NO: 48 - protein, 7 aa, synthetic construct
  REGION 1..7: note = COV2-2952 CDRH2
IYSGGST

SEQ ID NO: 49 - protein, 11 aa, synthetic construct
  REGION 1..11: note = COV2-2952 CDRH3
ARDLVTYGLDV

SEQ ID NO: 50 - protein, 8 aa, synthetic construct
  REGION 1..8: note = COV2-2514 CDRH1
GFIFDDYD

SEQ ID NO: 51 - protein, 8 aa, synthetic construct
  REGION 1..8: note = COV2-2514 CDRH2
INWNGGST

SEQ ID NO: 52 - protein, 22 aa, synthetic construct
  REGION 1..22: note = COV2-2514 CDRH3
AVIMSPIPRYSGYDWAGDAFDI

SEQ ID NO: 53 - protein, 8 aa, synthetic construct
  REGION 1..8: note = COV2-2391 CDRH1
GYTFGSFD

SEQ ID NO: 54 - protein, 8 aa, synthetic construct
  REGION 1..8: note = COV2-2391 CDRH2
MNSNSGNT

SEQ ID NO: 55 - protein, 16 aa, synthetic construct
  REGION 1..16: note = COV2-2391 CDRH3
ARMRSGWPTHGRPDDF

SEQ ID NO: 56 - protein, 8 aa, synthetic construct
  REGION 1..8: note = COV2-3025 CDRH1
GFTFMSSA

SEQ ID NO: 57 - protein, 8 aa, synthetic construct
  REGION 1..8: note = COV2-3025 CDRH2
IVIGSGNT

SEQ ID NO: 58 - protein, 16 aa, synthetic construct
  REGION 1..16: note = COV2-3025 CDRH3
AAPYCSSISCNDGFDI

SEQ ID NO: 59 - protein, 8 aa, synthetic construct
  REGION 1..8: note = COV2-2196 CDRH1
GFTFMSSA

SEQ ID NO: 60 - protein, 8 aa, synthetic construct
  REGION 1..8: note = COV2-2196 CDRH2
IVIGSGNT

SEQ ID NO: 61 - protein, 16 aa, synthetic construct
  REGION 1..16: note = COV2-2196 CDRH3
AAPYCSSISCNDGFDI

SEQ ID NO: 62 - protein, 8 aa, synthetic construct
  REGION 1..8: note = COV2-2094 CDRH1
GFIFDDYD

SEQ ID NO: 63 - protein, 8 aa, synthetic construct
  REGION 1..8: note = COV2-2094 CDRH2
INWNGGST

SEQ ID NO: 64 - protein, 22 aa, synthetic construct
  REGION 1..22: note = COV2-2094 CDRH3
AVIMSPIPRYSGYDWAGDAFDI

SEQ ID NO: 65 - protein, 8 aa, synthetic construct
  REGION 1..8: note = COV2-2096 CDRH1
GYTFGSFD

SEQ ID NO: 66 - protein, 8 aa, synthetic construct
  REGION 1..8: note = COV2-2096 CDRH2
MNSNSGNT

SEQ ID NO: 67 - protein, 16 aa, synthetic construct
  REGION 1..16: note = COV2-2096 CDRH3
ARMRSGWPTHGRPDDF

SEQ ID NO: 68 - protein, 8 aa, synthetic construct
  REGION 1..8: note = COV2-2130 CDRH1
GFTFRDVW

SEQ ID NO: 69 - protein, 10 aa, synthetic construct
  REGION 1..10: note = COV2-2130 CDRH2
IKSKIDGGTT

SEQ ID NO: 70 - protein, 22 aa, synthetic construct
  REGION 1..22: note = COV2-2130 CDRH3
TTAGSYYYDTVGPGLPEGKFDY

SEQ ID NO: 71 - protein, 6 aa, synthetic construct
  REGION 1..6: note = COV2-2165 CDRL1
QGISNY

SEQ ID NO: 72 - skipped

SEQ ID NO: 73 - protein, 9 aa, synthetic construct
  REGION 1..9: note = COV2-2165 CDRL3
QLLNSHPLT

SEQ ID NO: 74 - protein, 7 aa, synthetic construct
  REGION 1..7: note = COV2-2838 CDRL1
QSVSSSY

SEQ ID NO: 75 - skipped

SEQ ID NO: 76 - protein, 10 aa, synthetic construct
  REGION 1..10: note = COV2-2838 CDRL3
QHYGSSRGWT

SEQ ID NO: 77 - protein, 6 aa, synthetic construct
  REGION 1..6: note = COV2-2952 CDRL1
QGISNY

SEQ ID NO: 78 - skipped

SEQ ID NO: 79 - protein, 9 aa, synthetic construct
  REGION 1..9: note = COV2-2952 CDRL3
QLLNSHPLT

SEQ ID NO: 80 - protein, 6 aa, synthetic construct
  REGION 1..6: note = COV2-2514 CDRL1
SLRSYY

SEQ ID NO: 81 - skipped

SEQ ID NO: 82 - protein, 11 aa, synthetic construct
  REGION 1..11: note = COV2-2514 CDRL3
NSRDSSGNAVV

SEQ ID NO: 83 - protein, 8 aa, synthetic construct
  REGION 1..8: note = COV2-2391 CDRL1
NSNIGSYT

SEQ ID NO: 84 - skipped

SEQ ID NO: 85 - protein, 11 aa, synthetic construct
  REGION 1..11: note = COV2-2391 CDRL3
AVWDDSLNGLV

SEQ ID NO: 86 - protein, 7 aa, synthetic construct
  REGION 1..7: note = COV2-3025 CDRL1
QSVSSSY

SEQ ID NO: 87 - skipped

SEQ ID NO: 88 - protein, 10 aa, synthetic construct
  REGION 1..10: note = COV2-3025 CDRL3
QHYGSSRGWT

SEQ ID NO: 89 - protein, 7 aa, synthetic construct
  REGION 1..7: note = COV2-2196 CDRL1
QSVSSSY

SEQ ID NO: 90 - skipped

SEQ ID NO: 91 - protein, 10 aa, synthetic construct
  REGION 1..10: note = COV2-2196 CDRL3
QHYGSSRGWT

SEQ ID NO: 92 - protein, 6 aa, synthetic construct
  REGION 1..6: note = COV2-2094 CDRL1
SLRSYY

SEQ ID NO: 93 - skipped

SEQ ID NO: 94 - protein, 11 aa, synthetic construct
  REGION 1..11: note = COV2-2094 CDRL3
NSRDSSGNAVV

SEQ ID NO: 95 - protein, 8 aa, synthetic construct
  REGION 1..8: note = COV2-2096 CDRL1
NSNIGSYT

SEQ ID NO: 96 - skipped

SEQ ID NO: 97 - protein, 11 aa, synthetic construct
  REGION 1..11: note = COV2-2096 CDRL3
AVWDDSLNGLV

SEQ ID NO: 98 - protein, 12 aa, synthetic construct
  REGION 1..12: note = COV2-2130 CDRL1
QSVLYSSNNKNY

SEQ ID NO: 99 - skipped

SEQ ID NO: 100 - protein, 8 aa, synthetic construct
  REGION 1..8: note = COV2-2130 CDRL3
QQYYSTLT

SEQ ID NO: 101 - protein, 5 aa, synthetic construct
  REGION 1..5: note = IGHV1-58 FR2-HCDR2
IGWIV

SEQ ID NO: 102 - skipped

SEQ ID NO: 103 - protein, 10 aa, synthetic construct
  REGION 1..10: note = IGHD2-2 HCDR3-FR4
GYCSSTSCYA

SEQ ID NO: 104 - protein, 10 aa, synthetic construct
  REGION 1..10: note = IGHD2-8 HCDR3-FR4
GYCTNGVCYA

SEQ ID NO: 105 - protein, 10 aa, synthetic construct
  REGION 1..10: note = IGHD2-15 HCDR3-FR4
GYCSGGSCYS

SEQ ID NO: 106 - protein, 6 aa, synthetic construct
  REGION 1..6: note = IGHJ3*02 HCDR3-FR4
DAFDIW

SEQ ID NO: 107 - protein, 6 aa, synthetic construct
  REGION 1..6: note = IGKV3-20 LCDR1-FR2
SSYLAW

SEQ ID NO: 108 - protein, 6 aa, synthetic construct
  REGION 1..6: note = IGKV3-20 LCDR3-FR4
QYGSSP

SEQ ID NO: 109 - protein, 4 aa, synthetic construct
  REGION 1..4: note = IGKJ1*01 LCDR3-FR4
WTFG

SEQ ID NO: 110 - protein, 5 aa, synthetic construct
  REGION 1..5: note = COV2-2196 FR2-HCDR2
IGWIV

SEQ ID NO: 111 - protein, 18 aa, synthetic construct
  REGION 1..18: note = COV2-2196 HCDR3-FR4
CAAPYCSSISCNDGFDIW

SEQ ID NO: 112 - protein, 6 aa, synthetic construct
  REGION 1..6: note = COV2-2196 LCDR1-FR2
SSYLAW

SEQ ID NO: 113 - protein, 11 aa, synthetic construct
  REGION 1..11: note = COV2-2196 LCDR3-FR4
HYGSSRGWTFG

SEQ ID NO: 114 - protein, 5 aa, synthetic construct
  REGION 1..5: note = COV2-2381 FR2-HCDR2
IGWIA

SEQ ID NO: 115 - protein, 18 aa, synthetic construct
  REGION 1..18: note = COV2-2381 HCDR3-FR4
CAAPYCSRTSCHDAFDIW

SEQ ID NO: 116 - protein, 6 aa, synthetic construct
  REGION 1..6: note = COV2-2381 LCDR1-FR2
SSYLAW

SEQ ID NO: 117 - protein, 11 aa, synthetic construct
  REGION 1..11: note = COV2-2381 LCDR3-FR4
HFGSSSQWTFG

SEQ ID NO: 118 - protein, 5 aa, synthetic construct
  REGION 1..5: note = COV2-2072 FR2-HCDR2
IGWIV

SEQ ID NO: 119 - protein, 18 aa, synthetic construct
  REGION 1..18: note = COV2-2072 HCDR3-FR4
CAAPHCNRTSCYDAFDLW

SEQ ID NO: 120 - protein, 6 aa, synthetic construct
  REGION 1..6: note = COV2-2072 LCDR1-FR2
SSYLGW

SEQ ID NO: 121 - protein, 10 aa, synthetic construct
  REGION 1..10: note = COV2-2072 LCDR3-FR4
QYGSSPWTFG

SEQ ID NO: 122 - protein, 5 aa, synthetic construct
  REGION 1..5: note = MnC5t2p1_G1 FR2-HCDR2
IGWIV

SEQ ID NO: 123 - protein, 18 aa, synthetic construct
  REGION 1..18: note = MnC5t2p1_G1 HCDR3-FR4
CAAPRCSGGSCYDGFDIW

SEQ ID NO: 124 - protein, 6 aa, synthetic construct
  REGION 1..6: note = MnC5t2p1_G1 LCDR1-FR2
SSYLAW

SEQ ID NO: 125 - protein, 10 aa, synthetic construct
  REGION 1..10: note = MnC5t2p1_G1 LCDR3-FR4
QYGSSPWTFG

SEQ ID NO: 126 - protein, 5 aa, synthetic construct
  REGION 1..5: note = HbnC3t1p2_C6 FR2-HCDR2
IGWIV

SEQ ID NO: 127 - protein, 18 aa, synthetic construct
  REGION 1..18: note = HbnC3t1p2_C6 HCDR3-FR4
CAAPYCSSTRCYDAFDIW

SEQ ID NO: 128 - protein, 6 aa, synthetic construct
  REGION 1..6: note = HbnC3t1p2_C6 LCDR1-FR2
SSYLAW

SEQ ID NO: 129 - protein, 10 aa, synthetic construct
  REGION 1..10: note = HbnC3t1p2_C6 LCDR3-FR4
QYGRSPWTFG

SEQ ID NO: 130 - protein, 5 aa, synthetic construct
  REGION 1..5: note = HbnC3t1p1_C6 FR2-HCDR2
IGWIV

SEQ ID NO: 131 - protein, 18 aa, synthetic construct
  REGION 1..18: note = HbnC3t1p1_C6 HCDR3-FR4
CAAPHCSSTICYDGFDIW

SEQ ID NO: 132 - protein, 6 aa, synthetic construct
  REGION 1..6: note = HbnC3t1p1_C6 LCDR1-FR2
SSYLAW

SEQ ID NO: 133 - protein, 10 aa, synthetic construct
  REGION 1..10: note = HbnC3t1p1_C6 LCDR3-FR4
QYGSSPWTFG

SEQ ID NO: 134 - protein, 5 aa, synthetic construct
  REGION 1..5: note = S2E12 FR2-HCDR2
VGWIV

SEQ ID NO: 135 - protein, 18 aa, synthetic construct
  REGION 1..18: note = S2E12 HCDR3-FR4
CASPYCSGGSCSDGFDIW

SEQ ID NO: 136 - protein, 6 aa, synthetic construct
  REGION 1..6: note = S2E12 LCDR1-FR2
SSYLAW

SEQ ID NO: 137 - protein, 11 aa, synthetic construct
  REGION 1..11: note = S2E12 LCDR3-FR4
QYVGLTGWTFG

SEQ ID NO: 138 - protein, 5 aa, synthetic construct
  REGION 1..5: note = COV107_1 FR2-HCDR2
IGWIV

SEQ ID NO: 139 - protein, 18 aa, synthetic construct
  REGION 1..18: note = COV107_1 HCDR3-FR4
CAAPHCSSTSCFDAFDIW

SEQ ID NO: 140 - protein, 6 aa, synthetic construct
  REGION 1..6: note = COV107_1 LCDR1-FR2
SSYLAW

SEQ ID NO: 141 - protein, 10 aa, synthetic construct
  REGION 1..10: note = COV107_1 LCDR3-FR4
QYGNSPWTFG

SEQ ID NO: 142 - protein, 5 aa, synthetic construct
  REGION 1..5: note = COV107_2 FR2-HCDR2
IGWIV

SEQ ID NO: 143 - protein, 18 aa, synthetic construct
  REGION 1..18: note = COV107_2 HCDR3-FR4
CAAPYCSGGSCSDAFDIW

SEQ ID NO: 144 - protein, 6 aa, synthetic construct
  REGION 1..6: note = COV107_2 LCDR1-FR2
SSYLAW

SEQ ID NO: 145 - protein, 10 aa, synthetic construct
  REGION 1..10: note = COV107_2 LCDR3-FR4
QYGSSPWTFG

SEQ ID NO: 146 - protein, 5 aa, synthetic construct
  REGION 1..5: note = COV72 FR2-HCDR2
IGWIV

SEQ ID NO: 147 - protein, 18 aa, synthetic construct
  REGION 1..18: note = COV72 HCDR3-FR4
CAAVDCNSTSCYDAFDIW

SEQ ID NO: 148 - protein, 6 aa, synthetic construct
  REGION 1..6: note = COV72 LCDR1-FR2
SSYLAW

SEQ ID NO: 149 - protein, 10 aa, synthetic construct
  REGION 1..10: note = COV72 LCDR3-FR4
QYDISPWTFG

SEQ ID NO: 150 - protein, 5 aa, synthetic construct
  REGION 1..5: note = COV21_1 FR2-HCDR2
IGWIV

SEQ ID NO: 151 - protein, 18 aa, synthetic construct
  REGION 1..18: note = COV21_1 HCDR3-FR4
CAAPHCSGGSCLDAFDIW

SEQ ID NO: 152 - protein, 6 aa, synthetic construct
  REGION 1..6: note = COV21_1 LCDR1-FR2
SSYLAW

SEQ ID NO: 153 - protein, 10 aa, synthetic construct
  REGION 1..10: note = COV21_1 LCDR3-FR4
QYGSSPWTFG

SEQ ID NO: 154 - protein, 5 aa, synthetic construct
  REGION 1..5: note = COV21_2 FR2-HCDR2
IGWIV

SEQ ID NO: 155 - protein, 18 aa, synthetic construct
  REGION 1..18: note = COV21_2 HCDR3-FR4
CAAPHCSGGSCYDAFDIW

SEQ ID NO: 156 - protein, 6 aa, synthetic construct
  REGION 1..6: note = COV21_2 LCDR1-FR2
SSYLAW

SEQ ID NO: 157 - protein, 10 aa, synthetic construct
  REGION 1..10: note = COV21_2 LCDR3-FR4
QYGSSPWTFG

SEQ ID NO: 158 - protein, 5 aa, synthetic construct
  REGION 1..5: note = COV57_1 FR2-HCDR2
IGWIV

SEQ ID NO: 159 - protein, 18 aa, synthetic construct
  REGION 1..18: note = COV57_1 HCDR3-FR4
CAANHCSGGSCYDGFDIW

SEQ ID NO: 160 - protein, 6 aa, synthetic construct
  REGION 1..6: note = COV57_1 LCDR1-FR2
SSYLAW

SEQ ID NO: 161 - protein, 10 aa, synthetic construct
  REGION 1..10: note = COV57_1 LCDR3-FR4
QYGSSPWMFG

SEQ ID NO: 162 - protein, 5 aa, synthetic construct
  REGION 1..5: note = COV57_2 FR2-HCDR2
IGWIV

SEQ ID NO: 163 - protein, 18 aa, synthetic construct
  REGION 1..18: note = COV57_2 HCDR3-FR4
CAAPYCSGGSCNDAFDIW

SEQ ID NO: 164 - protein, 6 aa, synthetic construct
  REGION 1..6: note = COV57_2 LCDR1-FR2
SSYLAW

SEQ ID NO: 165 - protein, 10 aa, synthetic construct
  REGION 1..10: note = COV57_2 LCDR3-FR4
QYGSSPWTFG

SEQ ID NO: 166 - protein, 129 aa, synthetic construct
  REGION 1..129: note = HIP1 HEAVY CHAIN
  SITE 81: note = MISC_FEATURE - X can be Met, Val
  SITE 100: note = MISC_FEATURE - X can be Trp, Ser, Arg
  SITE 101: note = MISC_FEATURE - X can be Asp, Arg, Val
  SITE 102: note = MISC_FEATURE - X can be Leu, Arg, Ala
  SITE 103: note = MISC_FEATURE - X can be Ala, Gly
  SITE 104: note = MISC_FEATURE - X can be Tyr, Ile
  SITE 107: note = MISC_FEATURE - X can be Val, Cys
  SITE 108: note = MISC_FEATURE - X can be Val, Tyr, Thr
  SITE 109: note = MISC_FEATURE - X can be Gly, Val
  SITE 110: note = MISC_FEATURE - X can be Asp, Val
  SITE 111: note = MISC_FEATURE - X can be Cys, Ala
  SITE 112: note = MISC_FEATURE - X can be Ser, Thr
  SITE 113: note = MISC_FEATURE - X can be Arg, His, Ala
QMQLVQSGPEVKKPGTSVKVSCKASGFTFTSSAVQWVRQARGQRLEWIGWIVVGSGNTNYAQKFQERVTITRDMSTSTAYXELSSLRSEDTAVYYCAAPXXXXXCGXXXXXXXDAFDIWGQGTMVTVSS

SEQ ID NO: 167 - protein, 128 aa, synthetic construct
  REGION 1..128: note = HIP2 HEAVY CHAIN
  SITE 3: note = misc_feature - X can be Gln, Pro
  SITE 4: note = misc_feature - X can be Leu, Arg
  SITE 34: note = misc_feature - X can be Met, Val
  SITE 100: note = misc_feature - X can be Gly, Asn, Asp, Gln, Thr, Ser, Leu, Arg
  SITE 101: note = misc_feature - X can be Pro, Gly, Leu, Ser, Val, Lys, Ala
  SITE 102: note = misc_feature - X can be Ser, Gly, Ile, Val, Arg, Pro, Ala, Met
  SITE 103: note = misc_feature - X can be Tyr, Leu, Ile, Arg, Asn, Ala
  SITE 104: note = misc_feature - X can be Cys, Ser, Val, Tyr
  SITE 105: note = misc_feature - X can be Ser, Arg, Val, Tyr, Met
  SITE 106: note = misc_feature - X can be Ser, Gly, Val, Cys
  SITE 107: note = misc_feature - X can be Gly, Thr
  SITE 108: note = misc_feature - X can be Ser, Gly, Val, Thr
  SITE 109: note = misc_feature - X can be Cys, Ala, Thr, Asp
  SITE 110: note = misc_feature - X can be Tyr, Arg, Phe, Pro, Thr
  SITE 111: note = misc_feature - X can be Ala, Pro, Gly, Val, Cys, Arg
  SITE 112: note = misc_feature - X can be Asp, Thr, Ser, Asn, Leu, Ile, Tyr, Pro
QMXXVQSGPEVKKPGTSVKVSCKASGFTFTSSAXQWVRQARGQRLEWIGWIVVGSGNTNYAQKFQERVTITRDMSTSTAYMELSSLRSEDTAVYYCAAPXXXXXXXXXXXXXDAFDIWGQGTMVTVSS

SEQ ID NO: 168 - protein, 129 aa, synthetic construct
  REGION 1..129: note = HIP3 HEAVY CHAIN
  SITE 3: note = misc_feature - X can be Gln, Pro
  SITE 34: note = misc_feature - X can be Met or Val
  SITE 35: note = misc_feature - X can be Gln, Arg
  SITE 43: note = misc_feature - X can be Gln, Arg
  SITE 100: note = misc_feature - X can be Tyr, Pro, Ala, Arg, Gly
  SITE 101: note = misc_feature - X can be Glu, Leu, Pro, Tyr, Ser
  SITE 102: note = misc_feature - X can be Gly, Val, Ser, Cys, Tyr
  SITE 103: note = misc_feature - X can be Cys, Asp, Val, Gln, Thr
  SITE 104: note = misc_feature - X can be Gly, Asn
  SITE 106: note = misc_feature - X can be Asp, Val
  SITE 108: note = misc_feature - X can be Tyr, Ala, His
  SITE 109: note = misc_feature - X can be Thr, Gln, Ser
  SITE 110: note = misc_feature - X can be Val, His
  SITE 111: note = misc_feature - X can be Thr, Arg
  SITE 112: note = misc_feature - X can be Ala, Pro
  SITE 113: note = misc_feature - X can be Leu, Phe, Ala, Gly, Asn
QMXLVQSGPEVKKPGTSVKVSCKASGFTFTSSAXXWVRQARGXRLEWIGWIVVGSGNTNYAQKFQERVTITRDMSTSTAYMELSSLRSEDTAVYYCAAPXXXXXGXCXXXXXXDAFDIWGQGTMVTVSS

SEQ ID NO: 169 - protein, 106 aa, synthetic construct
  REGION 1..106: note = CORD HEAVY CHAIN
  SITE 19: note = misc_feature - X can be Arg, Leu
  SITE 78: note = misc_feature - X can be Val, Glu, Gly
  SITE 79: note = misc_feature - X can be Pro, Gly, or His
  SITE 80: note = misc_feature - X can be Cys, Ile, Tyr
  SITE 81: note = misc_feature - X can be Ser, Cys, Val
  SITE 85: note = misc_feature - X can be Cys, Ser, Val
  SITE 86: note = misc_feature - X can be Tyr, Ser, Val
  SITE 87: note = misc_feature - X can be Ser, Thr, Val
  SITE 88: note = misc_feature - X can be Tyr, Ala, Ser
  SITE 89: note = misc_feature - X can be Ser, Ala, Cys
  SITE 90: note = misc_feature - X can be Asp, Tyr
KASGFTFTSSAVQWVRQAXGQRLEWIGWIVVGSGNTNYAQKFQERVTITRDMSTSTAYMELSSLRSEDTAVYYCAAPXXXXGGSXXXXXXDAFDIWGQGTMVTVSS

SEQ ID NO: 170 - protein, 109 aa, synthetic construct
  REGION 1..109: note = HIP1 LIGHT CHAIN
  SITE 97: note = misc_feature - X can be Pro, Leu, Ser, Thr
EIVLTQSPGTLSLSPGERATLSCRASQSVSSSYLAWYQQKPGQAPRLLIYGASSRATGIPDRFSGSGSGTDFTLTISRLEPEDFAVYYCQQYGSSPXWTFGQGTKVEIK

SEQ ID NO: 171 - protein, 109 aa, synthetic construct; identical to SEQ ID NO: 170
  REGION 1..109: note = HIP2 LIGHT CHAIN
  SITE 97: note = misc_feature - X can be Pro, Leu, Ser, Thr

SEQ ID NO: 172 - protein, 109 aa, synthetic construct; identical to SEQ ID NO: 170
  REGION 1..109: note = HIP3 LIGHT CHAIN
  SITE 97: note = misc_feature - X can be Pro, Leu, Ser, Thr

SEQ ID NO: 173 - protein, 108 aa, synthetic construct
  REGION 1..108: note = HIP1 Light Chain
EIVLTQSPGTLSLSPGERATLSCRASQSVSSSYLAWYQQKPGQAPRLLIYGASSRATGIPDRFSGSGSGTDFTLTISRLEPEDFAVYYCQQYGSSPWTFGQGTKVEIK

SEQ ID NO: 174 - protein, 109 aa, synthetic construct
  REGION 1..109: note = HIP1 Light Chain
EIVLTQSPGTLSLSPGERATLSCRASQSVSSSYLAWYQQKPGQAPRLLIYGASSRATGIPDRFSGSGSGTDFTLTISRLEPEDFAVYYCQQYGSSPPWTFGQGTKVEIK

SEQ ID NO: 175 - protein, 108 aa, synthetic construct
  REGION 1..108: note = HIP1 Light Chain
EIVLTQSPGTLSLSPGERATLSCRASQSVSSSYLAWYQQKPGQAPRLLIYGASSRATGIPDRFSGSGSGTDFTLTISRLEPEDFAVYYCQQYGSSLWTFGQGTKVEIK

SEQ ID NO: 176 - protein, 108 aa, synthetic construct
  REGION 1..108: note = HIP1 Light Chain
EIVLTQSPGTLSLSPGERATLSCRASQSVSSSYLAWYQQKPGQAPRLLIYGASSRATGIPDRFSGSGSGTDFTLTISRLEPEDFAVYYCQQYGSSSWTFGQGTKVEIK

SEQ ID NO: 177 - protein, 109 aa, synthetic construct
  REGION 1..109: note = HIP1 Light Chain
EIVLTQSPGTLSLSPGERATLSCRASQSVSSSYLAWYQQKPGQAPRLLIYGASSRATGIPDRFSGSGSGTDFTLTISRLEPEDFAVYYCQQYGSSPTWTFGQGTKVEIK

SEQ ID NO: 178 - protein, 108 aa, synthetic construct; identical to SEQ ID NO: 173
  REGION 1..108: note = HIP2 Light Chain

SEQ ID NO: 179 - protein, 108 aa, synthetic construct; identical to SEQ ID NO: 175
  REGION 1..108: note = HIP2 Light Chain

SEQ ID NO: 180 - protein, 109 aa, synthetic construct; identical to SEQ ID NO: 174
  REGION 1..109: note = HIP2 Light Chain

SEQ ID NO: 181 - protein, 108 aa, synthetic construct; identical to SEQ ID NO: 176
  REGION 1..108: note = HIP2 Light Chain

SEQ ID NO: 182 - protein, 109 aa, synthetic construct; identical to SEQ ID NO: 177
  REGION 1..109: note = HIP2 Light Chain

SEQ ID NO: 183 - protein, 108 aa, synthetic construct; identical to SEQ ID NO: 173
  REGION 1..108: note = HIP3 Light Chain

SEQ ID NO: 184 - protein, 108 aa, synthetic construct; identical to SEQ ID NO: 175
  REGION 1..108: note = HIP3 Light Chain

SEQ ID NO: 185 - protein, 109 aa, synthetic construct; identical to SEQ ID NO: 174
  REGION 1..109: note = HIP3 Light Chain

SEQ ID NO: 186 - protein, 108 aa, synthetic construct; identical to SEQ ID NO: 176
  REGION 1..108: note = HIP3 Light Chain

SEQ ID NO: 187 - protein, 109 aa, synthetic construct; identical to SEQ ID NO: 177
  REGION 1..109: note = HIP3 Light Chain